European Patent Specification EP 3 715 458 B1, published February 28, 2024. Title: H7 AVIAN INFLUENZA VACCINE STRAIN WHICH DIFFERENTIATES INFECTED FROM VACCINATED ANIMALS, PREPARATION METHOD THEREFOR, AND APPLICATION. Applicant: Song, Jiasheng. Application PCT/CN2018/089525. The sequence listing filed with the application follows.

SEQUENCE LISTING (7 sequences)

SEQ ID NO: 1 - protein, 407 aa, artificial sequence
  an extracellular region amino acid sequence
VQAVNHSAAKGVTLLLPEPEWTYPRLSCPGSTFQKALLISPHRFGEIKGNSAPLIIREPFIACGPTECKHFALTHYAAQPGGYYNGTREDRNKLRHLISVKLGKIPTVENSIFHMAAWSGSACHDGKEWTYIGVDGPDSNALLKIKYGEAYTDTYHSYAKNILRTQESACNCIGGDCYLMITDGPASGVSECRFLKIREGRIIKEIFPTGRVKHTEECTCGFASNKTIECACRDNRYTAKRPFVKLNVETDTAEIRLMCTETYLDTPRPNDGSITGPCESDGDKGSGGIKGGFVHQRMASKIGRWYSRTMSKTKRMGMGLYVKYDGDPWTDSEALALSGVMVSMEEPGWYSFGFEIKDKKCDVPCIGIEMVHDGGKTTWHSAATAIYCLMGSGQLLWDTVTGVDMAL

SEQ ID NO: 2 - DNA, 1224 bp, artificial sequence
  the sequence containing type B NA extracellular region
gttcaggctgtaaatcattctgcagcaaaaggggtgacacttcttctcccagaaccggaatggacataccctcgtttatcttgcccgggctcaacctttcagaaagcactcctaattagcccccatagattcggagaaatcaaaggaaactcagctcccttgataataagggaaccttttattgcttgtggaccaacggaatgcaaacactttgctctaacccattatgcagctcaaccagggggatactacaatggaacaagagaagacagaaacaagctgaggcatctaatttcagtcaaattgggcaaaatcccaacagtagaaaactccattttccacatggcagcttggagcgggtccgcatgccatgatggtaaagaatggacatatatcggagttgatggccccgacagtaatgcattgctcaaaataaaatatggagaagcatatactgacacataccattcctatgcaaaaaacatcctaaggacacaagaaagtgcctgcaattgcatcgggggagattgttatcttatgataactgatggcccagcttcaggggttagtgaatgcagattccttaagattcgagagggcagaataataaaagaaatatttccaacaggaagagtaaaacatactgaggaatgcacatgcggatttgccagcaacaaaaccatagaatgtgcttgtagagataaccgttacacagcaaaaagaccctttgtcaaattaaatgtggagactgatacagcggaaataagattgatgtgcacagagacttatttggacacccccagaccaaatgatggaagcataacagggccttgcgaatctgatggggacaaagggagtggaggcatcaagggaggatttgttcatcaaagaatggcatccaagattggaaggtggtactctcgaacgatgtctaaaaccaaaagaatggggatgggactgtatgtaaaatatgatggagacccatggactgacagtgaagcccttgctcttagtggagtaatggtttcaatggaagaacctggttggtattcctttggcttcgaaataaaagataagaaatgtgatgtcccctgtattgggatagaaatggtacatgatggtgggaaaacgacttggcactcagcagcaacagccatttattgtttaatgggctcaggacaattgctgtgggacactgtcacaggtgttgatatggctctgtaa

SEQ ID NO: 3 - DNA, 203 bp, artificial sequence
  5'-end packaging signal sequence
agcaaaagcaggggtttaaaatgaatccaaatcagaaaataataaccattggatcaatctgtctggtagtcggactaattagcctaatattgcaaatagggaatataatctcaatatggattagccattcaattcaaactggaagtcaaaaccatactggaatatgcaaccaaaacatcattacctataaaaatagcacctgg

SEQ ID NO: 4 - DNA, 185 bp, artificial sequence
  3'-end packaging signal sequence
gaggccgtgcttctgggttgaattaatcaggggacgacctaaagaaaaaacaatctggactagtgcgagcagcatttctttttgtggcgtgaatagtgatactgtagattggtcttggccagacggtgctgagttgccattcagcattgacaagtagtctgttcaaaaaactccttgtttctact

SEQ ID NO: 5 - DNA, 890 bp, artificial sequence
  the nucleotide sequence of DeltaNS
agcaaaagcagggtgacaaaaacataatggatccaaacactgtgtcaagctttcaggtagattgctttctttggcatgtccgcaaacgagttgcagaccaagaactaggcgatgccccattccttgatcggcttcgccgagatcagaaatccctaagaggaaggggcagtactctcggtctggacatcaagacagccacacgtgctggaaagcagatagtggagcggattctgaaagaagaatccgatgaggcacttaaaatgaccatggcctctgtacctgcgtcgcgttacctaactgacatgactcttgaggaaatgtcatgataatggtccatgctcatacccaagcagaaagtggcaggccctctttgtatcagaatggaccaggcgatcatggataagaacatcatactgaaagcgaacttcagtgtgatttttgaccggctggagactctaatattgctaagggctttcaccgaagagggagcaattgttggcgaaatttcaccattgccttctcttccaggacatactgctgaggatgtcaaaaatgcagttggagtcctcatcggaggacttgaatggaatgataacacagttcgagtctctgaaactctacagagattcgcttggagaagcagtaatgagaatgggagacctccactcactccaaaacagaaacgagaaatggcgggaacaattaggtcagaagtttgaagaaataagatggttgattgaagaagtgagacacaaactgaagataacagagaatagttttgagcaaataacatttatgcaagccttacatctattgcttgaagtggagcaagagataagaactttctcgtttcagcttatttagtactaaaaaacacccttgtttctact

SEQ ID NO: 6 - protein, 407 aa, artificial sequence
  the extracellular region protein amino acid sequence
VQAVNRSATKGVTLLLPEPEWTYPRLSCPGSTFQKALLISPHRFGETKGNSAPLIIREPFIACGPNECKHFALTHYAAQPGGYYNGTRGDRNKLRHLISVKLGKIPTVENSIFHMAAWSGSACHDGKEWTYIGVDGPDNNALLKVKYGEAYTDTYHSYANKILRTQESACNCIGGNCYLMITDGSASGVSECRFLKIREGRIIKEIFPTGRVKHTEECTCGFASNKTIECACRDNSYTAKRPFVKLNVETDTAEIRLMCTDTYLDTPRPNDGSITGPCESNGDKGSGGIKGGFVHQRMESKIGRWYSRTMSKTERMGMGLYVKYDGDPWADSDALAFSGVMVSMKEPGWYSFGFEIKDKKCDVPCIGIEMVHDGGKETWHSAATAIYCLMGSGQLLWDTVTGVDMAL

SEQ ID NO: 7 - DNA, 1224 bp, artificial sequence
  the DNA sequence for coding the extracellular region protein amino acid sequence
gttcaggctgtgaaccgttctgcaacaaaaggggtgacacttcttctcccagaaccggagtggacatacccgcgtttatcttgcccgggctcaacctttcagaaagcactcctaattagccctcatagattcggagaaaccaaaggaaactcagctcccttgataataagggaaccttttattgcttgtggaccaaatgaatgcaaacactttgctctaacccattatgcagcccaaccagggggatactacaatggaacaagaggagacagaaacaagctgaggcatctaatttcagtcaaattgggcaaaatcccaacagtagaaaactccattttccacatggcagcatggagcgggtccgcgtgccatgatggtaaggaatggacatatatcggagttgatggccctgacaataatgcattgctcaaagtaaaatatggagaagcatatactgacacataccattcctatgcaaacaaaatcctaagaacacaagaaagtgcctgcaattgcatcgggggaaattgttatcttatgataactgatggctcagcttcaggtgttagtgaatgcagatttcttaagattcgagagggccgaataataaaagaaatatttccaacaggaagagtaaaacacactgaggaatgcacatgcggatttgccagcaataaaaccatagaatgtgcctgtagagataacagttacacagcaaaaagaccttttgtcaaattaaacgtggagactgatacagcagaaataagattgatgtgcacagatacttatttggacacccccagaccaaacgatggaagcataacaggcccttgtgaatctaatggggacaaagggagtggaggcatcaagggaggatttgttcatcaaagaatggaatccaagattggaaggtggtactctcgaacgatgtctaaaactgaaaggatggggatgggactgtatgtcaagtatgatggagacccatgggctgacagtgatgccctagcttttagtggagtaatggtttcaatgaaagaacctggttggtactcctttggcttcgaaataaaagataagaaatgcgatgtcccctgtattgggatagagatggtacatgatggtggaaaagagacttggcactcagcagcaacagccatttactgtttaatgggctcaggacagctgctgtgggacactgtcacaggtgttgacatggctctgtaa